European Patent Application EP 4 674 984 A1, published January 7, 2026. Title: COMPOSITIONS. Applicant: CPTx GmbH. The sequence listing filed with the application follows.

SEQUENCE LISTING (331 sequences)

SEQ ID NO: 1 - DNA, 6105 bp, synthetic construct
  source 1..6105: mol_type = other DNA
cgagtctctaccacagcatatgtgaccccgggcgggccctcagatgccatctggtgctactgtttcatggagaggagggtctccaggtgacgtgccgtggcgccgatgagtcaaaaggcacaagcagaaatcatatgactatggccgcctgaatcccccgtcacgaaccggtagcatcaacccagttgacagcttctgaccttccaacacttaacaggccagcgcagtaggcggcgtcttcacagtccctaagagccaaacctctagtggggagctgcaccagagttcctcggatcgctgagcgccctgtagcggcgcattaagcgcggcgggtgtggtggttacgcgcagcgtgaccgctacacttgccagcgccctagcgcccgctcctttcgctttcttcccttcctttctcgccacgttcgccggctttccccgtcaagctctaaatcgggggctccctttagggttccgatttagtgctttacggcacctcgaccccaaaaaacttgattagggtgatggttcacgtagtgggccatcgccctgatagacggtttttcgccctttgacgttggagtccacgttctttaatagtggactcttgttccaaactggaacaacactcaaccctatctcggtccaagtctattagcctagctccttgcccctttttgtgaaacaaattttatcgaaagaacttcgagcaattcccacatgctctcgtactttgggttacacacgcttggtcatcgttcgcccatacagacatttgcagcccgcatgtcctgggaacatccgctgtcggcaaagccggctgagcgattcaatacccgactcccggggcataacgggctaatcgggacgcacgtcgcgctaggtttgaggtcgatctttccgagaagctatatagtacggcctccggaccaagatacgcggtggactgataatgatgggcgaccctgccttatgcaacgacaccgcgaggctcgcaaggaatatttcttgatccattcggttctacatagagatttactcgacggtccacctacctgtacaatctaactacgtttagacttgtaagcgtgagacgatatcactggcttagttaattgaacgccactagatcagtgattgtcagcactcaccccaatgcttttcggggaaatgtgcgcggaaccttgatcgggcacgtaagaggttccaactttcaccataatgaaataagatcactaccgggcgtattttttgagttatcgagattttcaggagctaaggaagctaaaatggagaaaaaaatcactggatataccaccgttgatatatcccaatggcatcgtaaagaacattttgaggcatttcagtcagttgctcaatgtacctataaccagaccgttcagctggatattacggcctttttaaagaccgtaaagaaaaataagcacaagttttatccggcctttattcacattcttgcccgcctgatgaatgctcatccggaatttcgtatggcaatgaaagacggtgagctggtgatatgggatagtgttcacccttgttacaccgttttccatgagcaaactgaaacgttttcatcgctctggagtgaataccacgacgatttccggcagtttctacacatatattcgcaagatgtggcgtgttacggtgaaaacctggcctatttccctaaagggtttattgagaatatgtttttcgtctcagccaatccctgggtgagtttcaccagttttgatttaaacgtggccaatatggacaacttcttcgcccccgttttcaccatgggcaaatattatacgcaaggcgacaaggtgctgatgccgctggcgattcaggttcatcatgccgtttgtgatggcttccatgtcggcagaatgcttaatgaattacaacagtactgcgatgagtggcagggcggggcgtaatttgatatcgagctcgcttggactcctgttgatagatccagtaatgacctcagaactccatctggatttgttcagaacgctcggttgccgccgggcgttttttattggtgagaatccaagcctcgagctgtcagaccaagtttactcatatatactttagattgatttaaaacttcatttttaatttaaaaggatctaggtgaagatcctttttgataatctcatgaccaaaatcccttaacgtgagttttcgttccactgagcgtcagaccccgtagaaaagatcaaaggatcttcttgagatcctttttttctgcgcgtaatctgctgcttgcaaacaaaaaaaccaccgctaccagcggtggtttgtttgccggatcaagagctaccaactctttttccgaaggtaactggcttcagcagagcgcagataccaaatactgttcttctagtgtagccgtagttaggccaccacttcaagaactctgtagcaccgcctacatacctcgctctgctaatcctgttaccagtggctgctgccagtggcgataagtcgtgtcttaccgggttggactcaagacgatagttaccggataaggcgcagcggtcgggctgaacggggggttcgtgcacacagcccagcttggagcgaacgacctacaccgaactgagatacctacagcgtgagctatgagaaagcgccacgcttcccgaagggagaaaggcggacaggtatccggtaagcggcagggtcggaacaggagagcgcacgagggagcttccagggggaaacgcctggtatctttatagtcctgtcgggtttcgccacctctgacttgagcgtcgatttttgtgatgctcgtcaggggggcggagcctatggaaaaacgccagcaacgcggcctttttacggttcctggccttttgctggccttttgctcacgaaattcacctcgaaagcaagctgataaaccgatacaattaaaggctccttttggagcctttttttttggagattttcaacgtgaaaaaattattattcgcaattcctttagttgttcctttctattctcactccgctgaaactgttgaaagttgtttagcaaaaccccatacagaaaattcatttactaacgtctggaaagacgacaaaactttagatcgttacgctaactatgagggctgtctgtggaatgctacaggcgttgtagtttgtactggtgacgaaactcagtgttacggtacatgggttcctattgggcttgctatccctgaaaatgagggtggtggctctgagggtggcggttctgagggtggcggttctgagggtggcggtactaaacctcctgagtacggtgatacacctattccgggctatacttatatcaaccctctcgacggcacttatccgcctggtactgagcaaaaccccgctaatcctaatccttctcttgaggagtctcagcctcttaatactttcatgtttcagaataataggttccgaaataggcagggggcattaactgtttatacgggcactgttactcaaggcactgaccccgttaaaacttattaccagtacactcctgtatcatcaaaagccatgtatgacgcttactggaacggtaaattcagagactgcgctttccattctggctttaatgaggatccattcgtttgtgaatatcaaggccaatcgtctgacctgcctcaacctcctgtcaatgctggcggcggctctggtggtggttctggtggcggctctgagggtggtggctctgagggtggcggttctgagggtggcggctctgagggaggcggttccggtggtggctctggttccggtgattttgattatgaaaagatggcaaacgctaataagggggctatgaccgaaaatgccgatgaaaacgcgctacagtctgacgctaaaggcaaacttgattctgtcgctactgattacggtgctgctatcgatggtttcattggtgacgtttccggccttgctaatggtaatggtgctactggtgattttgctggctctaattcccaaatggctcaagtcggtgacggtgataattcacctttaatgaataatttccgtcaatatttaccttccctccctcaatcggttgaatgtcgcccttttgtctttggcgctggtaaaccatatgaattttctattgattgtgacaaaataaacttattccgtggtgtctttgcgtttcttttatatgttgccacctttatgtatgtattttctacgtttgctaacatactgcgtaataaggagtcttaatcatgccagttcttttgggttaagtaactaaggagctttaactcctactttcatacgccaccgcacagacttcattgaccacgtatctgagactccttgtaaactgactactccagctccatcaacaatcttgaagaagttctatccgatcacggttatcgcgagtcttagcgtagccaatgctgggccgtagcgtctacttaacggaaagaagggtgaaagctgccacagaaaataaattactatttacatttgtaagacaaagttagtatggttaaatactggcttagtctgcgggaaacttagccatacgacttggtttgcctatcgttacagcgtacgacccgttcaccaatcgcatttgcgatgcagataacaactcggacgaagtaaccacggagtatcctatctcttacgagtgttattctcattataaagtgcattggcagggggtgtgcgggtatactaaacgtaataagggattaccatgaaggtaaatgttcaggacaactctgtgtattgcgttaggatagcggaaaaactgcgcgtatgtggtaccagcacagaggatcgtcgcaagtgtcaagcctggggcacgactcttcgctctgctgtcaagatatttgcaccggaaatgcagcaccttaaaggataaacatagtagctgattctctgaagtcccagaagcagtaaagatcgaagtttgcagaatgccataccgtcccagataaacgtattggtgattcggtcattaaggaaatccagcatttgttcccgcaaccatctctgtacgagtattgttcttctttacgatccgaagaaggcctcgtcacgatgagatatcatagcttagattcacgtcattttacaattattcgcaagaacatgtgggccttctcccgccctcttccggaaatgacaacgtcggccagcattctatggatatccgtcacactaccgtcacctcttcgccgttagatggcactgctattcccgatttacaagcttcacgggcgcaatatggccctgagttgttttgggcgagtacgcgagcgtaaaatatatcgatcgcagatctctacgatcgggtcgtgtgaaccgcaccctataatacgttccaacttccaatagcacttcagactttccggcccacgaagaccttaatagcgtcgcatgcggcatgcaagtcacgctaaccgcacgattgctcatatccaatgcgcgtgcgacacgggattattgttagaaactctaagtgagcctctatcctccccttctgcacttatcgtgatttagttttgtggacgatctcgaccacgcagcctttaccgatggcgcagaaacactgacgctaatctcaggttccaaggcggaactagaaccagtaaaagcatgtagcccccaggatataaacgcgaaaccctgcggtgcttgcgcacgttctacgtgaccggtcatcaaggagccctggcggctatgtgttggccgggtcctaagatagggctggtctaggaagccgttctgttcacgccctatgtgagtcgttactgcaggattgcgcgcgcggctcgttgtcgcagatccactctacacccgaagttgcattagccggcgacatatcagcgctcagacagtgtgaacttcagccagatggtactccatgataataatggtacgcgttgagccgagacgtacatccattggcaagctagctcaggggctgggtttttctgttaagtttgatgagacagtgtgcatacgagatacccagtcccgtataccgaaccgtgaagggactccctgtcctgaatcatcgcgaattccaggttatcggttaccagtctggcaggcatcccactc

SEQ ID NO: 2 - DNA, 8064 bp, synthetic construct
  source 1..8064: mol_type = other DNA
tgatagacggtttttcgccctttgacgttggagtccacgttctttaatagtggactcttgttccaaactggaacaacactcaaccctatctcgggctattcttttgatttataagggattttgccgatttcggaaccaccatcaaacaggattttcgcctgctggggcaaaccagcgtggaccgcttgctgcaactctctcagggccaggcggtgaagggcaatcagctgttgcccgtctcactggtgaaaagaaaaaccaccctggcgcccaatacgcaaaccgcctctccccgcgcgttggccgattcattaatgcagctggcacgacaggtttcccgactggaaagcgggcagtgagcgcaacgcaattaatgtgagttagctcactcattaggcaccccaggctttacactttatgcttccggctcgtatgttgtgtggaattgtgagcggataacaatttcacacaggaaacagctatgaccatgattacgaattcgagctcggtacccggggatcctcaactgtgaggaggctcacggacgcgaagaacaggcacgcgtgctggcagaaacccccggtatgaccgtgaaaacggcccgccgcattctggccgcagcaccacagagtgcacaggcgcgcagtgacactgcgctggatcgtctgatgcagggggcaccggcaccgctggctgcaggtaacccggcatctgatgccgttaacgatttgctgaacacaccagtgtaagggatgtttatgacgagcaaagaaacctttacccattaccagccgcagggcaacagtgacccggctcataccgcaaccgcgcccggcggattgagtgcgaaagcgcctgcaatgaccccgctgatgctggacacctccagccgtaagctggttgcgtgggatggcaccaccgacggtgctgccgttggcattcttgcggttgctgctgaccagaccagcaccacgctgacgttctacaagtccggcacgttccgttatgaggatgtgctctggccggaggctgccagcgacgagacgaaaaaacggaccgcgtttgccggaacggcaatcagcatcgtttaactttacccttcatcactaaaggccgcctgtgcggctttttttacgggatttttttatgtcgatgtacacaaccgcccaactgctggcggcaaatgagcagaaatttaagtttgatccgctgtttctgcgtctctttttccgtgagagctatcccttcaccacggagaaagtctatctctcacaaattccgggactggtaaacatggcgctgtacgtttcgccgattgtttccggtgaggttatccgttcccgtggcggctccacctctgaaagcttggcactggccgtcgttttacaacgtcgtgactgggaaaaccctggcgttacccaacttaatcgccttgcagcacatccccctttcgccagctggcgtaatagcgaagaggcccgcaccgatcgcccttcccaacagttgcgcagcctgaatggcgaatggcgctttgcctggtttccggcaccagaagcggtgccggaaagctggctggagtgcgatcttcctgaggccgatactgtcgtcgtcccctcaaactggcagatgcacggttacgatgcgcccatctacaccaacgtgacctatcccattacggtcaatccgccgtttgttcccacggagaatccgacgggttgttactcgctcacatttaatgttgatgaaagctggctacaggaaggccagacgcgaattatttttgatggcgttcctattggttaaaaaatgagctgatttaacaaaaatttaatgcgaattttaacaaaatattaacgtttacaatttaaatatttgcttatacaatcttcctgtttttggggcttttctgattatcaaccggggtacatatgattgacatgctagttttacgattaccgttcatcgattctcttgtttgctccagactctcaggcaatgacctgatagcctttgtagatctctcaaaaatagctaccctctccggcattaatttatcagctagaacggttgaatatcatattgatggtgatttgactgtctccggcctttctcacccttttgaatctttacctacacattactcaggcattgcatttaaaatatatgagggttctaaaaatttttatccttgcgttgaaataaaggcttctcccgcaaaagtattacagggtcataatgtttttggtacaaccgatttagctttatgctctgaggctttattgcttaattttgctaattctttgccttgcctgtatgatttattggatgttaatgctactactattagtagaattgatgccaccttttcagctcgcgccccaaatgaaaatatagctaaacaggttattgaccatttgcgaaatgtatctaatggtcaaactaaatctactcgttcgcagaattgggaatcaactgttatatggaatgaaacttccagacaccgtactttagttgcatatttaaaacatgttgagctacagcattatattcagcaattaagctctaagccatccgcaaaaatgacctcttatcaaaaggagcaattaaaggtactctctaatcctgacctgttggagtttgcttccggtctggttcgctttgaagctcgaattaaaacgcgatatttgaagtctttcgggcttcctcttaatctttttgatgcaatccgctttgcttctgactataatagtcagggtaaagacctgatttttgatttatggtcattctcgttttctgaactgtttaaagcatttgagggggattcaatgaatatttatgacgattccgcagtattggacgctatccagtctaaacattttactattaccccctctggcaaaacttcttttgcaaaagcctctcgctattttggtttttatcgtcgtctggtaaacgagggttatgatagtgttgctcttactatgcctcgtaattccttttggcgttatgtatctgcattagttgaatgtggtattcctaaatctcaactgatgaatctttctacctgtaataatgttgttccgttagttcgttttattaacgtagatttttcttcccaacgtcctgactggtataatgagccagttcttaaaatcgcataaggtaattcacaatgattaaagttgaaattaaaccatctcaagcccaatttactactcgttctggtgtttctcgtcagggcaagccttattcactgaatgagcagctttgttacgttgatttgggtaatgaatatccggttcttgtcaagattactcttgatgaaggtcagccagcctatgcgcctggtctgtacaccgttcatctgtcctctttcaaagttggtcagttcggttcccttatgattgaccgtctgcgcctcgttccggctaagtaacatggagcaggtcgcggatttcgacacaatttatcaggcgatgatacaaatctccgttgtactttgtttcgcgcttggtataatcgctgggggtcaaagatgagtgttttagtgtattcttttgcctctttcgttttaggttggtgccttcgtagtggcattacgtattttacccgtttaatggaaacttcctcatgaaaaagtctttagtcctcaaagcctctgtagccgttgctaccctcgttccgatgctgtctttcgctgctgagggtgacgatcccgcaaaagcggcctttaactccctgcaagcctcagcgaccgaatatatcggttatgcgtgggcgatggttgttgtcattgtcggcgcaactatcggtatcaagctgtttaagaaattcacctcgaaagcaagctgataaaccgatacaattaaaggctccttttggagccttttttttggagattttcaacgtgaaaaaattattattcgcaattcctttagttgttcctttctattctcactccgctgaaactgttgaaagttgtttagcaaaatcccatacagaaaattcatttactaacgtctggaaagacgacaaaactttagatcgttacgctaactatgagggctgtctgtggaatgctacaggcgttgtagtttgtactggtgacgaaactcagtgttacggtacatgggttcctattgggcttgctatccctgaaaatgagggtggtggctctgagggtggcggttctgagggtggcggttctgagggtggcggtactaaacctcctgagtacggtgatacacctattccgggctatacttatatcaaccctctcgacggcacttatccgcctggtactgagcaaaaccccgctaatcctaatccttctcttgaggagtctcagcctcttaatactttcatgtttcagaataataggttccgaaataggcagggggcattaactgtttatacgggcactgttactcaaggcactgaccccgttaaaacttattaccagtacactcctgtatcatcaaaagccatgtatgacgcttactggaacggtaaattcagagactgcgctttccattctggctttaatgaggatttatttgtttgtgaatatcaaggccaatcgtctgacctgcctcaacctcctgtcaatgctggcggcggctctggtggtggttctggtggcggctctgagggtggtggctctgagggtggcggttctgagggtggcggctctgagggaggcggttccggtggtggctctggttccggtgattttgattatgaaaagatggcaaacgctaataagggggctatgaccgaaaatgccgatgaaaacgcgctacagtctgacgctaaaggcaaacttgattctgtcgctactgattacggtgctgctatcgatggtttcattggtgacgtttccggccttgctaatggtaatggtgctactggtgattttgctggctctaattcccaaatggctcaagtcggtgacggtgataattcacctttaatgaataatttccgtcaatatttaccttccctccctcaatcggttgaatgtcgcccttttgtctttggcgctggtaaaccatatgaattttctattgattgtgacaaaataaacttattccgtggtgtctttgcgtttcttttatatgttgccacctttatgtatgtattttctacgtttgctaacatactgcgtaataaggagtcttaatcatgccagttcttttgggtattccgttattattgcgtttcctcggtttccttctggtaactttgttcggctatctgcttacttttcttaaaaagggcttcggtaagatagctattgctatttcattgtttcttgctcttattattgggcttaactcaattcttgtgggttatctctctgatattagcgctcaattaccctctgactttgttcagggtgttcagttaattctcccgtctaatgcgcttccctgtttttatgttattctctctgtaaaggctgctattttcatttttgacgttaaacaaaaaatcgtttcttatttggattgggataaataatatggctgtttattttgtaactggcaaattaggctctggaaagacgctcgttagcgttggtaagattcaggataaaattgtagctgggtgcaaaatagcaactaatcttgatttaaggcttcaaaacctcccgcaagtcgggaggttcgctaaaacgcctcgcgttcttagaataccggataagccttctatatctgatttgcttgctattgggcgcggtaatgattcctacgatgaaaataaaaacggcttgcttgttctcgatgagtgcggtacttggtttaatacccgttcttggaatgataaggaaagacagccgattattgattggtttctacatgctcgtaaattaggatgggatattatttttcttgttcaggacttatctattgttgataaacaggcgcgttctgcattagctgaacatgttgtttattgtcgtcgtctggacagaattactttaccttttgtcggtactttatattctcttattactggctcgaaaatgcctctgcctaaattacatgttggcgttgttaaatatggcgattctcaattaagccctactgttgagcgttggctttatactggtaagaatttgtataacgcatatgatactaaacaggctttttctagtaattatgattccggtgtttattcttatttaacgccttatttatcacacggtcggtatttcaaaccattaaatttaggtcagaagatgaaattaactaaaatatatttgaaaaagttttctcgcgttctttgtcttgcgattggatttgcatcagcatttacatatagttatataacccaacctaagccggaggttaaaaaggtagtctctcagacctatgattttgataaattcactattgactcttctcagcgtcttaatctaagctatcgctatgttttcaaggattctaagggaaaattaattaatagcgacgatttacagaagcaaggttattcactcacatatattgatttatgtactgtttccattaaaaaaggtaattcaaatgaaattgttaaatgtaattaattttgttttcttgatgtttgtttcatcatcttcttttgctcaggtaattgaaatgaataattcgcctctgcgcgattttgtaacttggtattcaaagcaatcaggcgaatccgttattgtttctcccgatgtaaaaggtactgttactgtatattcatctgacgttaaacctgaaaatctacgcaatttctttatttctgttttacgtgcaaataattttgatatggtaggttctaacccttccattattcagaagtataatccaaacaatcaggattatattgatgaattgccatcatctgataatcaggaatatgatgataattccgctccttctggtggtttctttgttccgcaaaatgataatgttactcaaacttttaaaattaataacgttcgggcaaaggatttaatacgagttgtcgaattgtttgtaaagtctaatacttctaaatcctcaaatgtattatctattgacggctctaatctattagttgttagtgctcctaaagatattttagataaccttcctcaattcctttcaactgttgatttgccaactgaccagatattgattgagggtttgatatttgaggttcagcaaggtgatgctttagatttttcatttgctgctggctctcagcgtggcactgttgcaggcggtgttaatactgaccgcctcacctctgttttatcttctgctggtggttcgttcggtatttttaatggcgatgttttagggctatcagttcgcgcattaaagactaatagccattcaaaaatattgtctgtgccacgtattcttacgctttcaggtcagaagggttctatctctgttggccagaatgtcccttttattactggtcgtgtgactggtgaatctgccaatgtaaataatccatttcagacgattgagcgtcaaaatgtaggtatttccatgagcgtttttcctgttgcaatggctggcggtaatattgttctggatattaccagcaaggccgatagtttgagttcttctactcaggcaagtgatgttattactaatcaaagaagtattgctacaacggttaatttgcgtgatggacagactcttttactcggtggcctcactgattataaaaacacttctcaggattctggcgtaccgttcctgtctaaaatccctttaatcggcctcctgtttagctcccgctctgattctaacgaggaaagcacgttatacgtgctcgtcaaagcaaccatagtacgcgccctgtagcggcgcattaagcgcggcgggtgtggtggttacgcgcagcgtgaccgctacacttgccagcgccctagcgcccgctcctttcgctttcttcccttcctttctcgccacgttcgccggctttccccgtcaagctctaaatcgggggctccctttagggttccgatttagtgctttacggcacctcgaccccaaaaaacttgatttgggtgatggttcacgtagtgggccatcgccc

SEQ ID NO: 3 - DNA, 56 bp, synthetic construct
  source 1..56: mol_type = other DNA
tcacatatgttggaaaacgtttacaggagttagcgtcatacatggctccggatgat

SEQ ID NO: 4 - DNA, 49 bp, synthetic construct
  source 1..49: mol_type = other DNA
taattgtaaaatgatttttgtgaatctcgtagagatctgttccaaaact

SEQ ID NO: 5 - DNA, 51 bp, synthetic construct
  source 1..51: mol_type = other DNA
tagaatggattgccttgagtaacagtgcccgtataaatttttagttaatgt

SEQ ID NO: 6 - DNA, 58 bp, synthetic construct
  source 1..58: mol_type = other DNA
ttgggaattgctgatatgagcaatctttctatcagttgcaaaatcttacacaagtgtt

SEQ ID NO: 7 - DNA, 54 bp, synthetic construct
  source 1..54: mol_type = other DNA
tgcggtggttcagaaaaatttaggattttggtcagtttaagcgcagtctctgat

SEQ ID NO: 8 - DNA, 61 bp, synthetic construct
  source 1..61: mol_type = other DNA
ttcaaacctttatgtctgtatgggcgtttcggctcaacgcgttttttccattattatcatt

SEQ ID NO: 9 - DNA, 58 bp, synthetic construct
  source 1..58: mol_type = other DNA
taacactgatttaagatttttgctgagacttgatagcaattaaaaaaaagaataggtt

SEQ ID NO: 10 - DNA, 77 bp, synthetic construct
  source 1..77: mol_type = other DNA
taagtttctgttccgccgtttttgcttattcccactattggactccttagttctttttatagggttttctagcttgt

SEQ ID NO: 11 - DNA, 55 bp, synthetic construct
  source 1..55: mol_type = other DNA
taaaatcattattggccatttcaagattttgttaggagttaaagctccttagttt

SEQ ID NO: 12 - DNA, 50 bp, synthetic construct
  source 1..50: mol_type = other DNA
tcgggggattttgggttgattcccggggttttgcctgccttgaaaacgtt

SEQ ID NO: 13 - DNA, 57 bp, synthetic construct
  source 1..57: mol_type = other DNA
ttcgtggtatttcgccccccgttcagcccgaccgcttcaccctcattgctaggcggt

SEQ ID NO: 14 - DNA, 46 bp, synthetic construct
  source 1..46: mol_type = other DNA
tctgacagcttttttgaggcttggttacatattttttctcaataat

SEQ ID NO: 15 - DNA, 50 bp, synthetic construct
  source 1..50: mol_type = other DNA
taaacactcctttttttttacgcagtatttctttagcgtttttcagactt

SEQ ID NO: 16 - protein, 57 aa, synthetic construct
TCTAAAGTTTGTTGGTATTTTTGGTATTACACGACTTTTGCTACAGTTACATAGGGT

SEQ ID NO: 17 - DNA, 54 bp, synthetic construct
  source 1..54: mol_type = other DNA
ttgccccgggagtcggttagtgctgtttatcagtttcactatcttgcatctgat

SEQ ID NO: 18 - DNA, 56 bp, synthetic construct
  source 1..56: mol_type = other DNA
tggctttatcagcttttttctatgtttgcgcccgttttttaagcttgtaaatcggt

SEQ ID NO: 19 - DNA, 58 bp, synthetic construct
  source 1..58: mol_type = other DNA
ttccaacccttatccggtattgtaggtcgttcgctccttaacgactctttttcaccgt

SEQ ID NO: 20 - DNA, 49 bp, synthetic construct
  source 1..49: mol_type = other DNA
tggccgcgtttcttcgggaagcgtggcgctttttttctcttaaaaggct

SEQ ID NO: 21 - DNA, 57 bp, synthetic construct
  source 1..57: mol_type = other DNA
ttgacggatttcggaagagggcgggagttccctgccattagtagtcattgcgtatgt

SEQ ID NO: 22 - DNA, 51 bp, synthetic construct
  source 1..51: mol_type = other DNA
tacatttaccttttttcatggtaatcccttattttatgcactttataatgt

SEQ ID NO: 23 - DNA, 50 bp, synthetic construct
  source 1..50: mol_type = other DNA
tttaggacccggccaacacatagccgccaggtttgtccgcttcgcagggt

SEQ ID NO: 24 - DNA, 60 bp, synthetic construct
  source 1..60: mol_type = other DNA
tgaataacactcgtatttctgcgccatcggtttttaaaggctgcgtggtcgagatcgtct

SEQ ID NO: 25 - DNA, 55 bp, synthetic construct
  source 1..55: mol_type = other DNA
taaaggatcttcaccttttttgatccttttaaattaaaaaagcttgttccttgct

SEQ ID NO: 26 - DNA, 54 bp, synthetic construct
  source 1..54: mol_type = other DNA
tccagaaccttaccctcagttatttgcccatggcaaaccatttttcgctggtat

SEQ ID NO: 27 - DNA, 56 bp, synthetic construct
  source 1..56: mol_type = other DNA
tatgattttcggcccattttctttcttcgctgtaatttgtcttacttaacctgagt

SEQ ID NO: 28 - DNA, 78 bp, synthetic construct
  source 1..78: mol_type = other DNA
tccatatcaccagcttattaagttggatttgatctagtggcgttcttcccgattagcccgttattgttccttggagtt

SEQ ID NO: 29 - DNA, 64 bp, synthetic construct
  source 1..64: mol_type = other DNA
taaagcattggggtgttgtattgaattttcactccttggtgtagattgatagagtccactattt

SEQ ID NO: 30 - DNA, 58 bp, synthetic construct
  source 1..58: mol_type = other DNA
ttacatacagattccaatgaaaccatccgttgtgcggttttagtctgaagtgcgaatt

SEQ ID NO: 31 - DNA, 56 bp, synthetic construct
  source 1..56: mol_type = other DNA
ttgagcaaaaggccagcttatagctcacgctgtagttttcctagaccagccctatt

SEQ ID NO: 32 - DNA, 56 bp, synthetic construct
  source 1..56: mol_type = other DNA
tcaggacatgcgggcttttttcaattagcgcgtttttcgtgcgtttaattaactat

SEQ ID NO: 33 - DNA, 60 bp, synthetic construct
  source 1..60: mol_type = other DNA
taagaacgtttcgtgaaccatttttcaccttgtatcttgttcccatcatttacaatcact

SEQ ID NO: 34 - DNA, 51 bp, synthetic construct
  source 1..51: mol_type = other DNA
tataagtgttgtttgcaattgaaaaagattatatatgagtaaccccactat

SEQ ID NO: 35 - DNA, 57 bp, synthetic construct
  source 1..57: mol_type = other DNA
tccccctgttgaaagtatttgtttcgtcttgcgaataataatttttttcgtaaaaat

SEQ ID NO: 36 - DNA, 48 bp, synthetic construct
  source 1..48: mol_type = other DNA
tgtagcgcgttacgaaaattattctcatttcaaaactttttgtccatt

SEQ ID NO: 37 - DNA, 41 bp, synthetic construct
  source 1..41: mol_type = other DNA
tgcattggcttttttcgctaccggaaacgtcattactggct

SEQ ID NO: 38 - DNA, 47 bp, synthetic construct
  source 1..47: mol_type = other DNA
taggaactttcacgttgtttttaaatctccattgcccaataggaact

SEQ ID NO: 39 - DNA, 55 bp, synthetic construct
  source 1..55: mol_type = other DNA
ttgtctggcgcgcgcaatcctgcagtttaagctgggttttgcgaatatatgaagt

SEQ ID NO: 40 - DNA, 55 bp, synthetic construct
  source 1..55: mol_type = other DNA
tgaacctgtttgaaacatttcctatttctttgacaggaggttgaggcaggtcagt

SEQ ID NO: 41 - DNA, 57 bp, synthetic construct
  source 1..57: mol_type = other DNA
tgccagtgattcgcccggtagttttttatcttatttcatttaggccggataaaactt

SEQ ID NO: 42 - DNA, 53 bp, synthetic construct
  source 1..53: mol_type = other DNA
tgatcaaggttagggtgaattagagcgatttagatttggggtcgaggtgccgt

SEQ ID NO: 43 - DNA, 72 bp, synthetic construct
  source 1..72: mol_type = other DNA
tattttagcttcctcaccgtctttcatttcaggcgggcaagaatgtgaataatttatggtgattgctcctgt

SEQ ID NO: 44 - DNA, 61 bp, synthetic construct
  source 1..61: mol_type = other DNA
tattattcttaatcgccattattctgccgacatggaagtttttcatcacaaacgatctcat

SEQ ID NO: 45 - DNA, 60 bp, synthetic construct
  source 1..60: mol_type = other DNA
tttattttgttacgcaaagtttgagccatttcaccattattggccggaattagcgtgact

SEQ ID NO: 46 - DNA, 47 bp, synthetic construct
  source 1..47: mol_type = other DNA
tctcagcgatttttccgaggaactcttcggtatactttttggactgt

SEQ ID NO: 47 - DNA, 43 bp, synthetic construct
  source 1..43: mol_type = other DNA
tctagggcgctggtataaaagaatttcacaatttaaagacaat

SEQ ID NO: 48 - DNA, 57 bp, synthetic construct
  source 1..57: mol_type = other DNA
tgtgcttatttttctttacggtctttaaaatttgtactcaaaaaatatttatcgtct

SEQ ID NO: 49 - DNA, 48 bp, synthetic construct
  source 1..48: mol_type = other DNA
tccgcctccctttgtatcggtttttttttcagcttgctttcagccact

SEQ ID NO: 50 - DNA, 58 bp, synthetic construct
  source 1..58: mol_type = other DNA
tggtctggttataggtacattctttacgatgccattgttatggtttattgcccccgat

SEQ ID NO: 51 - DNA, 47 bp, synthetic construct
  source 1..47: mol_type = other DNA
ttgtactggtaataagttttttctgctttgcagcagattttggtcat

SEQ ID NO: 52 - DNA, 58 bp, synthetic construct
  source 1..58: mol_type = other DNA
ttgacgagcttgtgcgctcttacgatctaaagttttgtttgtatgggttggacggtat

SEQ ID NO: 53 - DNA, 68 bp, synthetic construct
  source 1..68: mol_type = other DNA
tatttaccgttagaaccgctttttgctcagtacccatttctgtggtatttgtgccttttgccatagtt

SEQ ID NO: 54 - DNA, 62 bp, synthetic construct
  source 1..62: mol_type = other DNA
tgaggtttcacttgtaaccgataaccagtttggaaatcgttttcagtttttgaatccccgat

SEQ ID NO: 55 - DNA, 56 bp, synthetic construct
  source 1..56: mol_type = other DNA
ttatattttttcattcaattaccgactttacaccacgaagtttttctgtgcggtgt

SEQ ID NO: 56 - DNA, 53 bp, synthetic construct
  source 1..53: mol_type = other DNA
taaaatgttttttgagcaactgactgaacgctcgcgtactcgcttcgatcgat

SEQ ID NO: 57 - DNA, 57 bp, synthetic construct
  source 1..57: mol_type = other DNA
tgaattatttcacacgacccgataatttaaggtgcttgagcgaagagtcgtgcccct

SEQ ID NO: 58 - DNA, 74 bp, synthetic construct
  source 1..74: mol_type = other DNA
tcgataggttgatactcttcgcaaatcacagagtttcctgctggttcaaatctgtttcgtgacgttttaaaggt

SEQ ID NO: 59 - DNA, 60 bp, synthetic construct
  source 1..60: mol_type = other DNA
ttgcgccttttggttgtagaaactgcctttaccttcgttgagactcgttctgttatcaat

SEQ ID NO: 60 - DNA, 61 bp, synthetic construct
  source 1..61: mol_type = other DNA
tagaagatcctttttttaacggttagcggggtttcaccctcattggaggtttagtaccgct

SEQ ID NO: 61 - DNA, 62 bp, synthetic construct
  source 1..62: mol_type = other DNA
tcatgttcttacggcgaagaggtgacggtagtgtttggcattcttcgtaaagaagaacacct

SEQ ID NO: 62 - DNA, 56 bp, synthetic construct
  source 1..56: mol_type = other DNA
ttgctaccggaaatttttgagcgggcgtttttagagttggaacccttaaatattct

SEQ ID NO: 63 - DNA, 54 bp, synthetic construct
  source 1..54: mol_type = other DNA
tgatagaggttatcacgataagtgcagaaacccagcccctgagttatcaaactt

SEQ ID NO: 64 - DNA, 48 bp, synthetic construct
  source 1..48: mol_type = other DNA
tactgtctcgagtgttgttcctttttgtttggaacatcaggacagggt

SEQ ID NO: 65 - DNA, 59 bp, synthetic construct
  source 1..59: mol_type = other DNA
tcacaaaactaattctcacttacagactaagccagtatttttttaaccatactaacttt

SEQ ID NO: 66 - DNA, 49 bp, synthetic construct
  source 1..49: mol_type = other DNA
tttgcatgcttgagtttctttgtattctgtggcagttttttttcaccct

SEQ ID NO: 67 - DNA, 46 bp, synthetic construct
  source 1..46: mol_type = other DNA
tgtcatttcttatccatagaatgctggagccgccgttaacgcctgt

SEQ ID NO: 68 - DNA, 61 bp, synthetic construct
  source 1..61: mol_type = other DNA
tcgcgatttgtggatctgcgacatcttctgtgtgcacgaactcagccggctttttcacact

SEQ ID NO: 69 - DNA, 64 bp, synthetic construct
  source 1..64: mol_type = other DNA
tggaacctaccaccagttattaagcttgcggcatttcgaaaactctttttcgtttttctacggt

SEQ ID NO: 70 - DNA, 54 bp, synthetic construct
  source 1..54: mol_type = other DNA
tagcggtcacgctgtttttgcgtaaccaccaggctcttagggattgagtgggat

SEQ ID NO: 71 - DNA, 67 bp, synthetic construct
  source 1..67: mol_type = other DNA
tgtataatttaaccgccattagagccacttcgccccccttagacttaccggataccttgctccttgt

SEQ ID NO: 72 - DNA, 55 bp, synthetic construct
  source 1..55: mol_type = other DNA
ttttaaattcgaagaagttggtgaaattttatatcctggggcgtttctcaagtct

SEQ ID NO: 73 - DNA, 57 bp, synthetic construct
  source 1..57: mol_type = other DNA
taaatctcgataacattgtgtcgttgcatttttaaggcagggtcgttgtccggaggt

SEQ ID NO: 74 - DNA, 45 bp, synthetic construct
  source 1..45: mol_type = other DNA
tttcgaggttttccgtttttgcaaatgaaaacgggggtttcaatt

SEQ ID NO: 75 - DNA, 77 bp, synthetic construct
  source 1..77: mol_type = other DNA
ttatcgccttgttcggtttactatcggaatttcgttgtatcaccttatataagtttagaaggatttaagggcatgat

SEQ ID NO: 76 - DNA, 67 bp, synthetic construct
  source 1..67: mol_type = other DNA
tggagctggttctcatcgctttcaaattacgccccgtcagatacgtggtttttcaatggaataagtt

SEQ ID NO: 77 - DNA, 48 bp, synthetic construct
  source 1..48: mol_type = other DNA
tcatgtaccgtttacgattggccttgttttttattcacaaacgaatgt

SEQ ID NO: 78 - DNA, 66 bp, synthetic construct
  source 1..66: mol_type = other DNA
tacgtggcgttggatatatttgagtaaatctctatgtagaacctatttagagccattccagcgcct

SEQ ID NO: 79 - DNA, 65 bp, synthetic construct
  source 1..65: mol_type = other DNA
ttcacgcttttatcgaccttcgtactatttcacaatttttaaggggcaaggtgcttcagcggatt

SEQ ID NO: 80 - DNA, 58 bp, synthetic construct
  source 1..58: mol_type = other DNA
tgaatagcagttttctgggacttcagagatttgacacttgcgacgattttgtcctgat

SEQ ID NO: 81 - DNA, 55 bp, synthetic construct
  source 1..55: mol_type = other DNA
tcgtacagttgaacttctttagacgctattaaggcccggcggcaaccgtgaagtt

SEQ ID NO: 82 - DNA, 53 bp, synthetic construct
  source 1..53: mol_type = other DNA
taaagtctgaacaaagtccaagaattcagcaccttgtcggatttaccctcagt

SEQ ID NO: 83 - DNA, 59 bp, synthetic construct
  source 1..59: mol_type = other DNA
taaagcactaaatcttcttgacggttgaccgtcttcaacggtttatatccagctgaact

SEQ ID NO: 84 - DNA, 53 bp, synthetic construct
  source 1..53: mol_type = other DNA
tgatcctcattaaagccttttttcaggtttcctcaagttatagcccgggctct

SEQ ID NO: 85 - DNA, 55 bp, synthetic construct
  source 1..55: mol_type = other DNA
tgcgggaattatttccttttcgatctttactgctttgccatctattttgcgaatt

SEQ ID NO: 86 - DNA, 55 bp, synthetic construct
  source 1..55: mol_type = other DNA
tcttaacccaaaataaaggtggcattaccagtagttttgggaatttttggaagtt

SEQ ID NO: 87 - DNA, 55 bp, synthetic construct
  source 1..55: mol_type = other DNA
tcatatgatgatctttttaagggattttttacgcgtttttttttttccgtcgagt

SEQ ID NO: 88 - DNA, 52 bp, synthetic construct
  source 1..52: mol_type = other DNA
tggatcaagtttaaagggattggcgatggttatgcgccgctacgtagaaaat

SEQ ID NO: 89 - DNA, 46 bp, synthetic construct
  source 1..46: mol_type = other DNA
tcattttcgaaatgtaaatagtttttaatttattatcagtagcgat

SEQ ID NO: 90 - DNA, 49 bp, synthetic construct
  source 1..49: mol_type = other DNA
tcaatagaaaattcatagaaaggaagggtttttagaaagcgttcgtgat

SEQ ID NO: 91 - DNA, 64 bp, synthetic construct
  source 1..64: mol_type = other DNA
tatgaccttttactggttctagttcttaatcgacgttttgccatcttttcgtattcgttaagtt

SEQ ID NO: 92 - DNA, 65 bp, synthetic construct
  source 1..65: mol_type = other DNA
tagaacagtattgctcttgatttcttgagttagggttgttgtactcattgagccaccaccctcat

SEQ ID NO: 93 - DNA, 56 bp, synthetic construct
  source 1..56: mol_type = other DNA
tccattagcaaggagactcgtttttgataaccgtgattattattcattaggccttt

SEQ ID NO: 94 - DNA, 48 bp, synthetic construct
  source 1..48: mol_type = other DNA
taagggcgattaatgcctctttggaacgtattataggtttcttcgtgt

SEQ ID NO: 95 - DNA, 47 bp, synthetic construct
  source 1..47: mol_type = other DNA
tgtctgacgctcagtggcgagctcgatattagtactgttgtaattct

SEQ ID NO: 96 - DNA, 58 bp, synthetic construct
  source 1..58: mol_type = other DNA
ttctgcgctttggccaggtagttcttgaagtgttttttggcctaactacccagggatt

SEQ ID NO: 97 - DNA, 45 bp, synthetic construct
  source 1..45: mol_type = other DNA
tgtcacctggagaccctcctctttttccatgaaaaagccggcgat

SEQ ID NO: 98 - DNA, 56 bp, synthetic construct
  source 1..56: mol_type = other DNA
taaaaggagcctttaacagttaaggaattttaccagtacaaactacttccagcatt

SEQ ID NO: 99 - DNA, 59 bp, synthetic construct
  source 1..59: mol_type = other DNA
tggtaacaggcacttctttctcctttgctggcgtttttccttacaactattagccgcct

SEQ ID NO: 100 - DNA, 58 bp, synthetic construct
  source 1..58: mol_type = other DNA
taactcagggccatattttttatccttttgctttttttgatatctcatttgctggtat

SEQ ID NO: 101 - DNA, 61 bp, synthetic construct
  source 1..61: mol_type = other DNA
tacctcttacgtgcccttgcattcattttgccatacgaaattttacggcacttgggcccgt

SEQ ID NO: 102 - DNA, 46 bp, synthetic construct
  source 1..46: mol_type = other DNA
tgtgtaacattttccgcgcacattccgccaccctcttttccagtat

SEQ ID NO: 103 - DNA, 54 bp, synthetic construct
  source 1..54: mol_type = other DNA
ttgagatgaagacaactttcaggcgttttgactcatcggcgcctttttgatgat

SEQ ID NO: 104 - DNA, 65 bp, synthetic construct
  source 1..65: mol_type = other DNA
tgtttacatttcggatattagatggttttgtgaacggttatctgcatttcgtggttattgatact

SEQ ID NO: 105 - DNA, 66 bp, synthetic construct
  source 1..66: mol_type = other DNA
tccgacgttttagccgccattttcaacagtttcactgttgttttgctaaacaacttagcattccat

SEQ ID NO: 106 - DNA, 73 bp, synthetic construct
  source 1..73: mol_type = other DNA
tggtaaatattgacggaaaggagtcttaaggcccattcttcggattttgcaaacttttaatgaccttccagat

SEQ ID NO: 107 - DNA, 46 bp, synthetic construct
  source 1..46: mol_type = other DNA
tcacatacgcgcagctttgacagcatttgcatttccggtgcatagt

SEQ ID NO: 108 - DNA, 58 bp, synthetic construct
  source 1..58: mol_type = other DNA
tccggaaccttccctcagatttatgcggagtgagaatttttagcgtatttcctgttct

SEQ ID NO: 109 - DNA, 57 bp, synthetic construct
  source 1..57: mol_type = other DNA
tatcctattgtcttttttatggctaagttcctgccattacgtttagtatacccgcgt

SEQ ID NO: 110 - DNA, 55 bp, synthetic construct
  source 1..55: mol_type = other DNA
ttttccccctggaattactataaattcttcgtccttcgccttggttgtcatagct

SEQ ID NO: 111 - DNA, 56 bp, synthetic construct
  source 1..56: mol_type = other DNA
ttaaatgaattttctttcgtctttttgaatcaccttgagttgttttgtcataatct

SEQ ID NO: 112 - DNA, 52 bp, synthetic construct
  source 1..52: mol_type = other DNA
tcagcgtagttagatttaggccgtattggtatatccagtgatttttttctct

SEQ ID NO: 113 - DNA, 70 bp, synthetic construct
  source 1..70: mol_type = other DNA
tgccctcatagttagaaaggattataggctcttcaccggaatttttcgcgtttctcacggctacactagt

SEQ ID NO: 114 - DNA, 67 bp, synthetic construct
  source 1..67: mol_type = other DNA
ttgccgggtggcgaaacccgacaggttgctccctcttatcacaaattaatacgttttgccaatactt

SEQ ID NO: 115 - DNA, 80 bp, synthetic construct
  source 1..80: mol_type = other DNA
tcgaacccaaagtacgatcggaaagttacaagtctttgcctcgcgttggtaggtgttggacagtatttttcaccagatgt

SEQ ID NO: 116 - DNA, 59 bp, synthetic construct
  source 1..59: mol_type = other DNA
tcgtaatatcttttattaaggttgtgcggttttcaccgtcttccgattgagggagggat

SEQ ID NO: 117 - DNA, 44 bp, synthetic construct
  source 1..44: mol_type = other DNA
tcaggcacaccctttttcccgttcgcatgcgacgtttttccgct

SEQ ID NO: 118 - DNA, 62 bp, synthetic construct
  source 1..62: mol_type = other DNA
gcagtagagtaggtagagattaggcattggctgagtttaggctacatgcggtcacgtagaat

SEQ ID NO: 119 - DNA, 80 bp, synthetic construct
  source 1..80: mol_type = other DNA
gcagtagagtaggtagagattaggcatattagcgtcagtgttttagagatagttcaaaccaattacgcaatagcgattgt

SEQ ID NO: 120 - DNA, 68 bp, synthetic construct
  source 1..68: mol_type = other DNA
gcagtagagtaggtagagattaggcatcgtgcgcaagattagctttttgagcgaggtatgtaggcggt

SEQ ID NO: 121 - DNA, 66 bp, synthetic construct
  source 1..66: mol_type = other DNA
gcagtagagtaggtagagattaggcatccccttatttttcatcggttcgtttaaattccaataaat

SEQ ID NO: 122 - DNA, 67 bp, synthetic construct
  source 1..67: mol_type = other DNA
gcagtagagtaggtagagattaggcattaacagaattgtatgcacttagggcgaattaacagggcgt

SEQ ID NO: 123 - DNA, 82 bp, synthetic construct
  source 1..82: mol_type = other DNA
gcagtagagtaggtagagattaggcatcagaatcattaaggggagtttcccgtgtcgcacgcgcattgcgattaacgtcaat

SEQ ID NO: 124 - DNA, 80 bp, synthetic construct
  source 1..80: mol_type = other DNA
gcagtagagtaggtagagattaggcatggtatctcagtttgcttgttagcattaaacgatagcagcaccttaacaataat

SEQ ID NO: 125 - DNA, 98 bp, synthetic construct
  source 1..98: mol_type = other DNA
gcagtagagtaggtagagattaggcatccaatggatgtacgtcttaacgatgattatttgtttttatagcttcgagcatgttcttgcgattaaaacat

SEQ ID NO: 126 - DNA, 64 bp, synthetic construct
  source 1..64: mol_type = other DNA
gcagtagagtaggtagagattaggcataccctttacacggtttttggtgcattgcctggaattt

SEQ ID NO: 127 - DNA, 78 bp, synthetic construct
  source 1..78: mol_type = other DNA
gcagtagagtaggtagagattaggcataccatctggctgaagttttgccgattaacttcgttccaccgcttctaatct

SEQ ID NO: 128 - DNA, 63 bp, synthetic construct
  source 1..63: mol_type = other DNA
gcagtagagtaggtagagattaggcatcgtgaacagaacggcttgtatctcattactggcagt

SEQ ID NO: 129 - DNA, 68 bp, synthetic construct
  source 1..68: mol_type = other DNA
gcagtagagtaggtagagattaggcattaacacgcttgggaaatattctgctgaattgctacttggtt

SEQ ID NO: 130 - DNA, 62 bp, synthetic construct
  source 1..62: mol_type = other DNA
gcagtagagtaggtagagattaggcatagtcccttttcacaacgagccagcgctgatatgtt

SEQ ID NO: 131 - DNA, 95 bp, synthetic construct
  source 1..95: mol_type = other DNA
gcagtagagtaggtagagattaggcatcgccggctaaagctaggcttttttatagacttggaccgagttcgataaattccaagcgtgtgtaccct

SEQ ID NO: 132 - DNA, 50 bp, synthetic construct
  source 1..50: mol_type = other DNA
taataagatgtttagtgaatcgccacgcaataataacggaataccttttt

SEQ ID NO: 133 - DNA, 46 bp, synthetic construct
  source 1..46: mol_type = other DNA
ataccagtgaaagattacagaccaggcgcttttttaggctggctga

SEQ ID NO: 134 - DNA, 43 bp, synthetic construct
  source 1..43: mol_type = other DNA
acaattttagattttgaagtttttcttaaatcctgatgcaaat

SEQ ID NO: 135 - DNA, 41 bp, synthetic construct
  source 1..41: mol_type = other DNA
ccttgatattcagagccgccaccagatttttccaccaccag

SEQ ID NO: 136 - DNA, 45 bp, synthetic construct
  source 1..45: mol_type = other DNA
gtgtagcgttttttcacgctgtgattgccgttccggggtgtacat

SEQ ID NO: 137 - DNA, 46 bp, synthetic construct
  source 1..46: mol_type = other DNA
caatcgcaagacaataggttggaaccttgcttctgtaaatcgtcgc

SEQ ID NO: 138 - DNA, 42 bp, synthetic construct
  source 1..42: mol_type = other DNA
acaaaaggagaaaactaataaggcagcgcgttgacagaatca

SEQ ID NO: 139 - DNA, 40 bp, synthetic construct
  source 1..40: mol_type = other DNA
tatcagggcggggaaaagcactaagagcgggattagacag

SEQ ID NO: 140 - DNA, 48 bp, synthetic construct
  source 1..48: mol_type = other DNA
catcgggaaaataaaggtttaacgaatagagataacccactagacttt

SEQ ID NO: 141 - DNA, 48 bp, synthetic construct
  source 1..48: mol_type = other DNA
aggcggtcagtattaaccgaacgatatctaaattagagccgtcggtgg

SEQ ID NO: 142 - DNA, 40 bp, synthetic construct
  source 1..40: mol_type = other DNA
aacggtgttacagagggcctgagagtttttttggagcaaa

SEQ ID NO: 143 - DNA, 47 bp, synthetic construct
  source 1..47: mol_type = other DNA
ccagaatggatagcagcaccattatcatatggcacgttgacgattaa

SEQ ID NO: 144 - DNA, 40 bp, synthetic construct
  source 1..40: mol_type = other DNA
ccgatttaaatcctgaaagagacgcagaaacagcggatca

SEQ ID NO: 145 - DNA, 39 bp, synthetic construct
  source 1..39: mol_type = other DNA
atgtgagcgagtggcggattgaccatcaaaaagattaag

SEQ ID NO: 146 - DNA, 40 bp, synthetic construct
  source 1..40: mol_type = other DNA
taggtcacgttggtgtctccgtggaacaggtcgattcacc

SEQ ID NO: 147 - DNA, 51 bp, synthetic construct
  source 1..51: mol_type = other DNA
cttgtagaacgtcagccgtctcgtctttgcccgaacggtaaccaccacacc

SEQ ID NO: 148 - DNA, 39 bp, synthetic construct
  source 1..39: mol_type = other DNA
caactttgttgacccccagcgattataccaagcgcgaaa

SEQ ID NO: 149 - DNA, 48 bp, synthetic construct
  source 1..48: mol_type = other DNA
tttgagagatatgtacgattcaaacaaggataaaaattttgcctttat

SEQ ID NO: 150 - DNA, 45 bp, synthetic construct
  source 1..45: mol_type = other DNA
ccaacaggaaatggattatttatgcggaacaagtttgagtaacat

SEQ ID NO: 151 - DNA, 40 bp, synthetic construct
  source 1..40: mol_type = other DNA
aaatcagagtaacagtagttacaatcagaaccggttgata

SEQ ID NO: 152 - DNA, 50 bp, synthetic construct
  source 1..50: mol_type = other DNA
caaaaggggagccagctggcgaaagggggatgtgtagaaaatacattttt

SEQ ID NO: 153 - DNA, 49 bp, synthetic construct
  source 1..49: mol_type = other DNA
tttttcaaaagaactggcagcaaacgctgcaaggaaatctccaaaaaaa

SEQ ID NO: 154 - DNA, 37 bp, synthetic construct
  source 1..37: mol_type = other DNA
aatgggaaccgtgcatctgccagtttgaggatgttta

SEQ ID NO: 155 - DNA, 42 bp, synthetic construct
  source 1..42: mol_type = other DNA
agtcacgacgttgtaaaacgacggtttttcagtgccaagctt

SEQ ID NO: 156 - DNA, 50 bp, synthetic construct
  source 1..50: mol_type = other DNA
attgagggagggacggaaacaatcggagttaagcaatccaaataagaaac

SEQ ID NO: 157 - DNA, 32 bp, synthetic construct
  source 1..32: mol_type = other DNA
tttttactggctcattaccagacgacgttttt

SEQ ID NO: 158 - DNA, 39 bp, synthetic construct
  source 1..39: mol_type = other DNA
cgatggcctttggggtcgaggtgttccacactgtgaaat

SEQ ID NO: 159 - DNA, 47 bp, synthetic construct
  source 1..47: mol_type = other DNA
accaccagagatagaacccttctgcattctggcaattcgacaacatt

SEQ ID NO: 160 - DNA, 47 bp, synthetic construct
  source 1..47: mol_type = other DNA
accctcaagaggctgagactcctaaacatgacagagccaataggaac

SEQ ID NO: 161 - DNA, 44 bp, synthetic construct
  source 1..44: mol_type = other DNA
ttttgcttgaatttacctttttttccagtaagcgtcatacatgg

SEQ ID NO: 162 - DNA, 40 bp, synthetic construct
  source 1..40: mol_type = other DNA
gagtgagaaaggccggaacattatgacccagcgcagtctc

SEQ ID NO: 163 - DNA, 38 bp, synthetic construct
  source 1..38: mol_type = other DNA
tcaaatatcaaaccctcaattttttaatatgtcatacc

SEQ ID NO: 164 - DNA, 33 bp, synthetic construct
  source 1..33: mol_type = other DNA
ccaccctcagaactttagcgtcatttttactgt

SEQ ID NO: 165 - DNA, 41 bp, synthetic construct
  source 1..41: mol_type = other DNA
ttttttaatttaggcagaaagtaccgtattaatagactacc

SEQ ID NO: 166 - DNA, 39 bp, synthetic construct
  source 1..39: mol_type = other DNA
atcgcctgtgttacttagccggagagagccaacggtgtc

SEQ ID NO: 167 - DNA, 48 bp, synthetic construct
  source 1..48: mol_type = other DNA
tccgcgacacggctggaggtgtccgcagcaccgtcaatagtttacaaa

SEQ ID NO: 168 - DNA, 45 bp, synthetic construct
  source 1..45: mol_type = other DNA
caacaatagcttatccggtattctccatattattttgcacccagc

SEQ ID NO: 169 - DNA, 37 bp, synthetic construct
  source 1..37: mol_type = other DNA
aatcggtttagccagcataattcgcgtctggaggctc

SEQ ID NO: 170 - DNA, 54 bp, synthetic construct
  source 1..54: mol_type = other DNA
tcgtcataaacatcccttactttttctggtgtgttcagcaaatcgttaacggca

SEQ ID NO: 171 - DNA, 55 bp, synthetic construct
  source 1..55: mol_type = other DNA
tagctctccagccttttaccatatcaaaccccgtactatgatgatggttatcatc

SEQ ID NO: 172 - DNA, 50 bp, synthetic construct
  source 1..50: mol_type = other DNA
agtcacaaaattaagcaataaagcttttttcagagcatatccaataaatc

SEQ ID NO: 173 - DNA, 49 bp, synthetic construct
  source 1..49: mol_type = other DNA
cttaattggcataaccacaatgacaacaaccaatcaaaaatcacgccat

SEQ ID NO: 174 - DNA, 57 bp, synthetic construct
  source 1..57: mol_type = other DNA
ttagcgtttttaacctccctaattttttttccagttacaaaataaacagaagaacgc

SEQ ID NO: 175 - DNA, 45 bp, synthetic construct
  source 1..45: mol_type = other DNA
aaaatctacgttaataaaacgatgggcttgagatggtactcatct

SEQ ID NO: 176 - DNA, 42 bp, synthetic construct
  source 1..42: mol_type = other DNA
cagagccacctaagtatagcccggaaacctgagcagaggcga

SEQ ID NO: 177 - DNA, 44 bp, synthetic construct
  source 1..44: mol_type = other DNA
tgacgctctttttatcgtctgccattgcatttttcaggaaaaac

SEQ ID NO: 178 - DNA, 46 bp, synthetic construct
  source 1..46: mol_type = other DNA
gaacattttttatttttgaggacagttgaacggggtcagcggttgc

SEQ ID NO: 179 - DNA, 47 bp, synthetic construct
  source 1..47: mol_type = other DNA
tttttttcttaccagtaacatagcatagtgaatttatcatgataaat

SEQ ID NO: 180 - DNA, 40 bp, synthetic construct
  source 1..40: mol_type = other DNA
aacaccggaatcataacggccaacgctaacgaccttttta

SEQ ID NO: 181 - DNA, 40 bp, synthetic construct
  source 1..40: mol_type = other DNA
ggtctggtcagcagctatagcccgaagagtccactattaa

SEQ ID NO: 182 - DNA, 40 bp, synthetic construct
  source 1..40: mol_type = other DNA
gatatattcggtcgctaaagacagtgtcaatcatctacaa

SEQ ID NO: 183 - DNA, 40 bp, synthetic construct
  source 1..40: mol_type = other DNA
ttgtataacagggagttcttaaacagcttgatcgcaactg

SEQ ID NO: 184 - DNA, 45 bp, synthetic construct
  source 1..45: mol_type = other DNA
aacataccattaattgcgttgccgggttagcgggccgttttcacg

SEQ ID NO: 185 - DNA, 55 bp, synthetic construct
  source 1..55: mol_type = other DNA
aatgaatttgtcgtctttccagattctgaataatggtttctccgtggtgaaggga

SEQ ID NO: 186 - DNA, 39 bp, synthetic construct
  source 1..39: mol_type = other DNA
gagattatttgcacggcacgtatgggatagcatgccccc

SEQ ID NO: 187 - DNA, 48 bp, synthetic construct
  source 1..48: mol_type = other DNA
attgctttatcgtaggaatcagggagccgtttttattttcatatccca

SEQ ID NO: 188 - DNA, 40 bp, synthetic construct
  source 1..40: mol_type = other DNA
tagcgtttgacatgcaatgcctgagtaatgtgaatatgat

SEQ ID NO: 189 - DNA, 46 bp, synthetic construct
  source 1..46: mol_type = other DNA
aaaactggtaataagttttaacggaacagttaaagcccaccaccct

SEQ ID NO: 190 - DNA, 49 bp, synthetic construct
  source 1..49: mol_type = other DNA
attacgcaaacgcaaccgaggaaatatttaacaacgccaacatgttttt

SEQ ID NO: 191 - DNA, 45 bp, synthetic construct
  source 1..45: mol_type = other DNA
gttaaataatcctgaatcttaaatacaaaagggcgacattcaacc

SEQ ID NO: 192 - DNA, 38 bp, synthetic construct
  source 1..38: mol_type = other DNA
aacgagtagatttagtacgaggcgatattcattaccca

SEQ ID NO: 193 - DNA, 47 bp, synthetic construct
  source 1..47: mol_type = other DNA
gtgcactctgtggtgggttttgcagtgtttttcgatttcggaaccta

SEQ ID NO: 194 - DNA, 53 bp, synthetic construct
  source 1..53: mol_type = other DNA
tacaggcaaggtcaattctactaattttttgtagtagtaaacgttaactagca

SEQ ID NO: 195 - DNA, 45 bp, synthetic construct
  source 1..45: mol_type = other DNA
tgttcttgggggtttctttttgccagcacactcaatccgccgggc

SEQ ID NO: 196 - DNA, 39 bp, synthetic construct
  source 1..39: mol_type = other DNA
gagagggtagctattacgctgaggtcaccctcagcagcg

SEQ ID NO: 197 - DNA, 48 bp, synthetic construct
  source 1..48: mol_type = other DNA
tttgcggatttttggcttagagcgttttatttttttcgagcttcaaag

SEQ ID NO: 198 - DNA, 45 bp, synthetic construct
  source 1..45: mol_type = other DNA
atcctcattaaaggcaggtcacattttcgttcataattatatttt

SEQ ID NO: 199 - DNA, 40 bp, synthetic construct
  source 1..40: mol_type = other DNA
caccaatgccaaaaactcatatattttaaaggaggttgag

SEQ ID NO: 200 - DNA, 39 bp, synthetic construct
  source 1..39: mol_type = other DNA
gtgtaaagaactcgtaatcatggtcctgagaaacgtgct

SEQ ID NO: 201 - DNA, 49 bp, synthetic construct
  source 1..49: mol_type = other DNA
aatcccttataaagtgagacgggcaacatttttctgattgcccttcacc

SEQ ID NO: 202 - DNA, 47 bp, synthetic construct
  source 1..47: mol_type = other DNA
gtgccggatgccatcccaccgtaacaaagctactaaagtcctttaat

SEQ ID NO: 203 - DNA, 37 bp, synthetic construct
  source 1..37: mol_type = other DNA
aactgatagccctaaaagtctttacaatatttttgaa

SEQ ID NO: 204 - DNA, 40 bp, synthetic construct
  source 1..40: mol_type = other DNA
ttgcaggccgcgcggggtttttcttttcaccatcaaaaga

SEQ ID NO: 205 - DNA, 44 bp, synthetic construct
  source 1..44: mol_type = other DNA
aattatttttcaccgtcacccggataacctcacaggggagccgc

SEQ ID NO: 206 - DNA, 48 bp, synthetic construct
  source 1..48: mol_type = other DNA
gcgtctttccagagccgacttgcgggaggatattctgtccagacgacg

SEQ ID NO: 207 - DNA, 47 bp, synthetic construct
  source 1..47: mol_type = other DNA
ggtaatgggtaaaggtttctttgctcggccaagctttcgcgcgtgcc

SEQ ID NO: 208 - DNA, 40 bp, synthetic construct
  source 1..40: mol_type = other DNA
agattaagtttccattaaacgggtctttttcatgaggaag

SEQ ID NO: 209 - DNA, 39 bp, synthetic construct
  source 1..39: mol_type = other DNA
ccggagacagtcaaatcaccatctaggtaaacccggttg

SEQ ID NO: 210 - DNA, 42 bp, synthetic construct
  source 1..42: mol_type = other DNA
ccagtcgggaaacctgtcgtttttgccagctgcattaatgaa

SEQ ID NO: 211 - DNA, 40 bp, synthetic construct
  source 1..40: mol_type = other DNA
cttatcattccaagaaaacaagcagtgcctaaccctgcat

SEQ ID NO: 212 - DNA, 38 bp, synthetic construct
  source 1..38: mol_type = other DNA
acagtatcggcctgccagttacgaggcatagtaagagc

SEQ ID NO: 213 - DNA, 48 bp, synthetic construct
  source 1..48: mol_type = other DNA
taggtgtatttttcaccgtactcactccggctagaacgcgtaaagtaa

SEQ ID NO: 214 - DNA, 55 bp, synthetic construct
  source 1..55: mol_type = other DNA
ttaaatccgctggcaatgaagggaagccgcacaggcggcagatgggcgcatcgta

SEQ ID NO: 215 - DNA, 45 bp, synthetic construct
  source 1..45: mol_type = other DNA
agggtgagaatgtttatttttctatattttcatttggtagataca

SEQ ID NO: 216 - DNA, 56 bp, synthetic construct
  source 1..56: mol_type = other DNA
catcggaaactaaagaaaaatacgtaatgccactacgaagcgattttaagattttt

SEQ ID NO: 217 - DNA, 45 bp, synthetic construct
  source 1..45: mol_type = other DNA
gctattaggtggcacaaagaattgctccttaccggaagtccccct

SEQ ID NO: 218 - DNA, 40 bp, synthetic construct
  source 1..40: mol_type = other DNA
ccccttataaaccatcgaatgtaatacttttgcgggagaa

SEQ ID NO: 219 - DNA, 44 bp, synthetic construct
  source 1..44: mol_type = other DNA
gccgcgcttaatgcgccgcttagaatcaatcggaacgtttcctg

SEQ ID NO: 220 - DNA, 56 bp, synthetic construct
  source 1..56: mol_type = other DNA
ataatacaaccgccacagaagataacttgtttttctgagtagaagaacttctttga

SEQ ID NO: 221 - DNA, 56 bp, synthetic construct
  source 1..56: mol_type = other DNA
ctttagtggcctccggccagagcacatccgaacaaactccgaacaaacaacaaccc

SEQ ID NO: 222 - DNA, 45 bp, synthetic construct
  source 1..45: mol_type = other DNA
gagtgaatgttatattttttactatattttaatggaaacagtaca

SEQ ID NO: 223 - DNA, 48 bp, synthetic construct
  source 1..48: mol_type = other DNA
agaaaagtgttttcccattcattaaagataataatttttttttaccag

SEQ ID NO: 224 - DNA, 40 bp, synthetic construct
  source 1..40: mol_type = other DNA
accagcttctgctccaataaattgtgtcgaaactgttgcc

SEQ ID NO: 225 - DNA, 37 bp, synthetic construct
  source 1..37: mol_type = other DNA
tttttaacggaaccagagccaccaagaaccgccaccc

SEQ ID NO: 226 - DNA, 47 bp, synthetic construct
  source 1..47: mol_type = other DNA
gcactccagccagctaatagcgagaggctttatcataaccctcgttt

SEQ ID NO: 227 - DNA, 47 bp, synthetic construct
  source 1..47: mol_type = other DNA
agccctcatgaagggttagaaccacagagagtcaaaaatcagagggt

SEQ ID NO: 228 - DNA, 38 bp, synthetic construct
  source 1..38: mol_type = other DNA
aaatcaatatatgtacaataaacaatttttatgttcag

SEQ ID NO: 229 - DNA, 32 bp, synthetic construct
  source 1..32: mol_type = other DNA
aagtttattcagtagcttcatcgggacgattg

SEQ ID NO: 230 - DNA, 47 bp, synthetic construct
  source 1..47: mol_type = other DNA
ggtctgagtaattttcccttagaatccttgaaataaagcctcatctt

SEQ ID NO: 231 - DNA, 32 bp, synthetic construct
  source 1..32: mol_type = other DNA
agggcgaaaaaccgtcaacttaaaaaggagcg

SEQ ID NO: 232 - DNA, 43 bp, synthetic construct
  source 1..43: mol_type = other DNA
atacactaaaacttaatttcatttttctttaatcattgggaag

SEQ ID NO: 233 - DNA, 34 bp, synthetic construct
  source 1..34: mol_type = other DNA
acacttgctttttaaaagaagttttcaggaagat

SEQ ID NO: 234 - DNA, 39 bp, synthetic construct
  source 1..39: mol_type = other DNA
aaagagtttttacagatgctaaaacgaaagaggcaaaag

SEQ ID NO: 235 - DNA, 36 bp, synthetic construct
  source 1..36: mol_type = other DNA
atacgtaaaagggaacctgaaataatagaatatctt

SEQ ID NO: 236 - DNA, 49 bp, synthetic construct
  source 1..49: mol_type = other DNA
ataaaagagtatgttatgattaagactccttagccgaacaaagtttttt

SEQ ID NO: 237 - DNA, 44 bp, synthetic construct
  source 1..44: mol_type = other DNA
gccgatttttttaagggattgctaaatttttaggagtttagaag

SEQ ID NO: 238 - DNA, 43 bp, synthetic construct
  source 1..43: mol_type = other DNA
accagtcccggaatttgaccgatctaaagtttttctgtatggg

SEQ ID NO: 239 - DNA, 47 bp, synthetic construct
  source 1..47: mol_type = other DNA
ccaataataagagcaatcagaggttaaatatttttttgacggaaatt

SEQ ID NO: 240 - DNA, 39 bp, synthetic construct
  source 1..39: mol_type = other DNA
aaatattcatttcataacggaacagagagtactaacaac

SEQ ID NO: 241 - DNA, 48 bp, synthetic construct
  source 1..48: mol_type = other DNA
aatatccagaacggtagtgaggcctgaggatcagaatgcgcctgcagc

SEQ ID NO: 242 - DNA, 40 bp, synthetic construct
  source 1..40: mol_type = other DNA
gaaacaatgaaatagctttttatagctatcttaccgaagc

SEQ ID NO: 243 - DNA, 48 bp, synthetic construct
  source 1..48: mol_type = other DNA
tcagtaccggattaggattagcggagcaatactcaaactatataatca

SEQ ID NO: 244 - DNA, 39 bp, synthetic construct
  source 1..39: mol_type = other DNA
ttattctgcaagagaaaggcggataagtgccgtgtcact

SEQ ID NO: 245 - DNA, 40 bp, synthetic construct
  source 1..40: mol_type = other DNA
aaacaactgaacaactaaaggaattgcgagtggcaaaatc

SEQ ID NO: 246 - DNA, 41 bp, synthetic construct
  source 1..41: mol_type = other DNA
gaatataggcattttcgagccagaacgctcaacagtttttt

SEQ ID NO: 247 - DNA, 46 bp, synthetic construct
  source 1..46: mol_type = other DNA
ttcagaaaacgagaatgactttttataacatcagttttttgagatt

SEQ ID NO: 248 - DNA, 57 bp, synthetic construct
  source 1..57: mol_type = other DNA
ggttgcttgatacaggagtgttacctacatttgagcggaacaattcatcaatggcaa

SEQ ID NO: 249 - DNA, 48 bp, synthetic construct
  source 1..48: mol_type = other DNA
tcattccaagaaccggcagacggtcaaagtacaacggagatttgtatc

SEQ ID NO: 250 - DNA, 42 bp, synthetic construct
  source 1..42: mol_type = other DNA
atagttagcgtaattgagccatttgggaattttttagagcca

SEQ ID NO: 251 - DNA, 45 bp, synthetic construct
  source 1..45: mol_type = other DNA
aacgatgccgcttattaattttaaaaagaaaccactttttagaag

SEQ ID NO: 252 - DNA, 47 bp, synthetic construct
  source 1..47: mol_type = other DNA
ggtttgccctttttagcaggcgaaaatcctaagccggcgaacgtggc

SEQ ID NO: 253 - DNA, 40 bp, synthetic construct
  source 1..40: mol_type = other DNA
tgcctgccttgctggtgctcatggttcctcgtacagggcg

SEQ ID NO: 254 - DNA, 49 bp, synthetic construct
  source 1..49: mol_type = other DNA
aatcaagcataggagcagcagcaaagcaacagtgccacgctttgaccat

SEQ ID NO: 255 - DNA, 39 bp, synthetic construct
  source 1..39: mol_type = other DNA
ttttttacataaaggtggcaacatgaagcttgctttcga

SEQ ID NO: 256 - DNA, 48 bp, synthetic construct
  source 1..48: mol_type = other DNA
gaggcgttctaatgcagaacgcgcattacctttgtaaatgtttcaatt

SEQ ID NO: 257 - DNA, 37 bp, synthetic construct
  source 1..37: mol_type = other DNA
tagcacgaccagtaatggcacagaatgcgcggcgtaa

SEQ ID NO: 258 - DNA, 38 bp, synthetic construct
  source 1..38: mol_type = other DNA
ctggtctgtccatcacttagtaatatttttcatcaaac

SEQ ID NO: 259 - DNA, 40 bp, synthetic construct
  source 1..40: mol_type = other DNA
tttaaccaataggttcaaatatcgaatattttttgcgccg

SEQ ID NO: 260 - DNA, 42 bp, synthetic construct
  source 1..42: mol_type = other DNA
ttttttaccagaaggaaaagacaccattactagagtgtgata

SEQ ID NO: 261 - DNA, 40 bp, synthetic construct
  source 1..40: mol_type = other DNA
aaaaggaaagggggtaatagtaaaggacgacgagtcagaa

SEQ ID NO: 262 - DNA, 40 bp, synthetic construct
  source 1..40: mol_type = other DNA
ttaaacagaactaatgaggtcattagctcaacatgtttta

SEQ ID NO: 263 - DNA, 46 bp, synthetic construct
  source 1..46: mol_type = other DNA
tcgccattcaggctgaccgataggttaaaatttaaattgcattaac

SEQ ID NO: 264 - DNA, 43 bp, synthetic construct
  source 1..43: mol_type = other DNA
caatcataagggaacccaatcccaattctgcgtttcgcaaatg

SEQ ID NO: 265 - DNA, 36 bp, synthetic construct
  source 1..36: mol_type = other DNA
ggaagcccgaaaaaaccaggcaaagggtccgcttct

SEQ ID NO: 266 - DNA, 48 bp, synthetic construct
  source 1..48: mol_type = other DNA
ttcgcctggcgcgcctcagacgatccagcgcacaagaaaagaaaaata

SEQ ID NO: 267 - DNA, 48 bp, synthetic construct
  source 1..48: mol_type = other DNA
aaaagaagattacatttaacaatttcatttgactgtttatattattca

SEQ ID NO: 268 - DNA, 42 bp, synthetic construct
  source 1..42: mol_type = other DNA
tttttagggcttaattgaatcatatgcgttatacaaattttt

SEQ ID NO: 269 - DNA, 48 bp, synthetic construct
  source 1..48: mol_type = other DNA
tagatttttacaaactcgtaacactgagtttccgccacccaatcgcgc

SEQ ID NO: 270 - DNA, 40 bp, synthetic construct
  source 1..40: mol_type = other DNA
ctgcggctggtatgagccgggtcaatcaccttaggaaggt

SEQ ID NO: 271 - DNA, 32 bp, synthetic construct
  source 1..32: mol_type = other DNA
ggcgcgagtggaagttaatatgcagctcattc

SEQ ID NO: 272 - DNA, 49 bp, synthetic construct
  source 1..49: mol_type = other DNA
gaataccaaccttttaccatgtacacaacgccccttgagcaaacaaata

SEQ ID NO: 273 - DNA, 44 bp, synthetic construct
  source 1..44: mol_type = other DNA
cgagggtagcaacggctcgcccacctgattttttataatgctgt

SEQ ID NO: 274 - DNA, 40 bp, synthetic construct
  source 1..40: mol_type = other DNA
agtttgccgtcaccagcaggtttaacgtcctatttatccc

SEQ ID NO: 275 - DNA, 42 bp, synthetic construct
  source 1..42: mol_type = other DNA
tataacagttgatgagaatcgatttttgaacggtaatcgtaa

SEQ ID NO: 276 - DNA, 32 bp, synthetic construct
  source 1..32: mol_type = other DNA
ttttcaaacaaaatcaccggaggtttagtacc

SEQ ID NO: 277 - DNA, 46 bp, synthetic construct
  source 1..46: mol_type = other DNA
aatttttgttaacgtggtgaatttaaaggccgctctaaatttaatg

SEQ ID NO: 278 - DNA, 46 bp, synthetic construct
  source 1..46: mol_type = other DNA
tagaacccaggaagaataatcagcgggatcaagagtcagatagctt

SEQ ID NO: 279 - DNA, 48 bp, synthetic construct
  source 1..48: mol_type = other DNA
agccgccgccaccctcccggaaccgcctccctaaatcataagttaatt

SEQ ID NO: 280 - DNA, 39 bp, synthetic construct
  source 1..39: mol_type = other DNA
accagtagcaccgtaatttgtcactaccgaccaaaagcc

SEQ ID NO: 281 - DNA, 48 bp, synthetic construct
  source 1..48: mol_type = other DNA
cgaaccagttgataagatcgtcatagtgaataaggcttgctcttgaca

SEQ ID NO: 282 - DNA, 47 bp, synthetic construct
  source 1..47: mol_type = other DNA
taacagtgcccgtataggtcagtgtgtagcattccacgataaaacag

SEQ ID NO: 283 - DNA, 44 bp, synthetic construct
  source 1..44: mol_type = other DNA
tcagatgcgctcactgtgagcctctgttatccctgagagagttg

SEQ ID NO: 284 - DNA, 47 bp, synthetic construct
  source 1..47: mol_type = other DNA
cagcggtgccggtgcctgagtgagccgagctcgaatggacattttca

SEQ ID NO: 285 - DNA, 38 bp, synthetic construct
  source 1..38: mol_type = other DNA
cggtgcgggacaacgccatcaaaatttcatcaacatta

SEQ ID NO: 286 - DNA, 49 bp, synthetic construct
  source 1..49: mol_type = other DNA
ttattacagtttttgtacaggacgttgtgaattaccttatggcaccaac

SEQ ID NO: 287 - DNA, 40 bp, synthetic construct
  source 1..40: mol_type = other DNA
atgatgaaacaaacatgtcgagaggccaccctaagtatta

SEQ ID NO: 288 - DNA, 47 bp, synthetic construct
  source 1..47: mol_type = other DNA
ctgaaaacatcgccattaaaaatacaccgccttgaaaaatctaaagc

SEQ ID NO: 289 - DNA, 36 bp, synthetic construct
  source 1..36: mol_type = other DNA
tcaataaccaggaggctatcaggtcattctttgagg

SEQ ID NO: 290 - DNA, 46 bp, synthetic construct
  source 1..46: mol_type = other DNA
tttttataaaaaccaattccggcactttacccttttttactattat

SEQ ID NO: 291 - DNA, 42 bp, synthetic construct
  source 1..42: mol_type = other DNA
ctcacagtaccgagtaaaagagtcagttttttggcaaatcaa

SEQ ID NO: 292 - DNA, 40 bp, synthetic construct
  source 1..40: mol_type = other DNA
taatcggctagcaagcgattttttaaattgcgacagcgcc

SEQ ID NO: 293 - DNA, 48 bp, synthetic construct
  source 1..48: mol_type = other DNA
cgcgtccgcccgctttgcctggccgctcacaaccgtgtttgatggtgg

SEQ ID NO: 294 - DNA, 61 bp, synthetic construct
  source 1..61: mol_type = other DNA
tcatttttgagcctttaattgtatcggtttatcaaatccattagcatagaaagttcaacag

SEQ ID NO: 295 - DNA, 38 bp, synthetic construct
  source 1..38: mol_type = other DNA
gaggcttggcaaatattcgcattattcaacgaaagcta

SEQ ID NO: 296 - DNA, 40 bp, synthetic construct
  source 1..40: mol_type = other DNA
ccagcattgccatcttgtcatagcgtttgaaaaatcaata

SEQ ID NO: 297 - DNA, 40 bp, synthetic construct
  source 1..40: mol_type = other DNA
gggcggttaagaatttttagcgatttctgctcatttgccg

SEQ ID NO: 298 - DNA, 48 bp, synthetic construct
  source 1..48: mol_type = other DNA
cagcagttagaacgtggattttttccaacgtcaattccgaaatcggca

SEQ ID NO: 299 - DNA, 48 bp, synthetic construct
  source 1..48: mol_type = other DNA
ctgactttgaaaagcctaatgccgattcaaccgttctagccagagccg

SEQ ID NO: 300 - DNA, 59 bp, synthetic construct
  source 1..59: mol_type = other DNA
tactgaacaccctggcattagagaaccatacggaaattgtttggattatacgattatca

SEQ ID NO: 301 - DNA, 38 bp, synthetic construct
  source 1..38: mol_type = other DNA
tcgcactcatcgagcgggtattagcataaacacccaaa

SEQ ID NO: 302 - DNA, 41 bp, synthetic construct
  source 1..41: mol_type = other DNA
tatcagaacataaaaacagggaagcaacaaagtgaaaatag

SEQ ID NO: 303 - DNA, 38 bp, synthetic construct
  source 1..38: mol_type = other DNA
tagaaaccaatcaatcctaattctgaacaacaaaatta

SEQ ID NO: 304 - DNA, 54 bp, synthetic construct
  source 1..54: mol_type = other DNA
gcaaattaaccgttgtctgcggcccccgggtactaactcagagccggaaaacct

SEQ ID NO: 305 - DNA, 46 bp, synthetic construct
  source 1..46: mol_type = other DNA
aagattagttgagatgaatatacatatagaaggataagtctacgat

SEQ ID NO: 306 - DNA, 41 bp, synthetic construct
  source 1..41: mol_type = other DNA
gaaacaatcctttaccgcgcccaatgtctttcaattgagct

SEQ ID NO: 307 - DNA, 46 bp, synthetic construct
  source 1..46: mol_type = other DNA
cgccagaatcatagctcctaaaggtcaagtttcactacgtcgggat

SEQ ID NO: 308 - DNA, 40 bp, synthetic construct
  source 1..40: mol_type = other DNA
tgctccaatactgcggacagatacataacgccccacattc

SEQ ID NO: 309 - DNA, 36 bp, synthetic construct
  source 1..36: mol_type = other DNA
tgaatgttccagcgttttttgtggtgcttattagac

SEQ ID NO: 310 - DNA, 51 bp, synthetic construct
  source 1..51: mol_type = other DNA
taagattgggcgtgccaacgagcatcagaggaattggctgaaccagaggtg

SEQ ID NO: 311 - DNA, 44 bp, synthetic construct
  source 1..44: mol_type = other DNA
tgcaagaacgagaagagtaacctgacgagaacaacataggaata

SEQ ID NO: 312 - DNA, 50 bp, synthetic construct
  source 1..50: mol_type = other DNA
agaaaggaaggcaaacgcggtctttggaacagatagggttgagtgtttat

SEQ ID NO: 313 - DNA, 43 bp, synthetic construct
  source 1..43: mol_type = other DNA
gaactgacccttcatctagtaaatactaacggaaacacctgtt

SEQ ID NO: 314 - DNA, 55 bp, synthetic construct
  source 1..55: mol_type = other DNA
agcaagcggtccacgcaaccgcaagaaccagggtggagaggcggtttgcgttact

SEQ ID NO: 315 - DNA, 58 bp, synthetic construct
  source 1..58: mol_type = other DNA
gcagtagagtaggtagagattaggcacacgggaagtgagagaaagaattgcgaaacgt

SEQ ID NO: 316 - DNA, 58 bp, synthetic construct
  source 1..58: mol_type = other DNA
gcagtagagtaggtagagattaggcaatattcctcgttagtacttttgattgacagac

SEQ ID NO: 317 - DNA, 50 bp, synthetic construct
  source 1..50: mol_type = other DNA
gcagtagagtaggtagagattaggcaggcgctagggcgctatgagcttga

SEQ ID NO: 318 - DNA, 58 bp, synthetic construct
  source 1..58: mol_type = other DNA
gcagtagagtaggtagagattaggcacgacataaaaaaatcccgtaaaaataaagtta

SEQ ID NO: 319 - DNA, 58 bp, synthetic construct
  source 1..58: mol_type = other DNA
gcagtagagtaggtagagattaggcagtcggatttatcatttcattggcaaggtcgta

SEQ ID NO: 320 - DNA, 67 bp, synthetic construct
  source 1..67: mol_type = other DNA
gcagtagagtaggtagagattaggcagcaaagcggattgcgtcaaatgctgactggatagcgtaatt

SEQ ID NO: 321 - DNA, 58 bp, synthetic construct
  source 1..58: mol_type = other DNA
gcagtagagtaggtagagattaggcaggtgccgggcctcttcgctattacagggcgat

SEQ ID NO: 322 - DNA, 59 bp, synthetic construct
  source 1..59: mol_type = other DNA
gcagtagagtaggtagagattaggcatttcagcgccttcctggtaccaaaaaaatcagc

SEQ ID NO: 323 - DNA, 58 bp, synthetic construct
  source 1..58: mol_type = other DNA
gcagtagagtaggtagagattaggcagttgggtaacgccaggaagcagatcgccaaag

SEQ ID NO: 324 - DNA, 26 bp, synthetic construct
  source 1..26: mol_type = other DNA
gcagtagagtaggtagagattaggca

SEQ ID NO: 325 - DNA, 26 bp, synthetic construct
  source 1..26: mol_type = other DNA
acggattagagatggatgagatgacg

SEQ ID NO: 326 - DNA, 26 bp, synthetic construct
  source 1..26: mol_type = other DNA
gtgtctggtatggtgctgggatcgtg

SEQ ID NO: 327 - DNA, 26 bp, synthetic construct
  source 1..26: mol_type = other DNA
tggtgctatgtgtctggtctgggtat

SEQ ID NO: 328 - DNA, 26 bp, synthetic construct
  source 1..26: mol_type = other DNA
gtgtgatgtggagtgaggtggaggtg

SEQ ID NO: 329 - DNA, 26 bp, synthetic construct
  source 1..26: mol_type = other DNA
agcagtagagtaggtagagattaggc

SEQ ID NO: 330 - DNA, 26 bp, synthetic construct
  source 1..26: mol_type = other DNA
agggattagagatggatgagatgacg

SEQ ID NO: 331 - DNA, 26 bp, synthetic construct
  source 1..26: mol_type = other DNA
gcagtagagtaggtagagattaggca